European Patent Application EP 4 302 776 A1, published January 10, 2024. Title: A combination therapy of an insulinotropic peptide and GLP-2 for preventing or treating short bowel syndrome. Applicant: HANMI PHARM. CO., LTD. The sequence listing filed with the application follows.

SEQUENCE LISTING (35 sequences)

SEQ ID NO: 1 - protein, 33 aa, Homo sapiens
HADGSFSDEMNTILDNLAARDFINWLIQTKITD

SEQ ID NO: 2 - protein, 34 aa, Artificial Sequence
  GLP-2 derivative
  MISC_FEATURE (1): Xaa is imidazoacetyldeshistidine
XGDGSFSDEMNTILDNLAARDFINWLIQTKITDC

SEQ ID NO: 3 - protein, 34 aa, Artificial Sequence
  GLP-2 derivative
  MISC_FEATURE (1): Xaa is imidazoacetyldeshistidine
XGDGSFSDEMNTILDNLAARDFINWLIQTKITDK

SEQ ID NO: 4 - protein, 34 aa, Artificial Sequence
  GLP-2 derivative
  MISC_FEATURE (1): Xaa is imidazoacetyldeshistidine
XGDGSFSDEMNTILDNLAARDFINWLIQTRITDK

SEQ ID NO: 5 - protein, 34 aa, Artificial Sequence
  GLP-2 derivative
  MISC_FEATURE (1): Xaa is imidazoacetyldeshistidine
  MISC_FEATURE (34): Xaa is 6-azidolysine
XGDGSFSDEMNTILDNLAARDFINWLIQTKITDX

SEQ ID NO: 6 - protein, 34 aa, Artificial Sequence
  GLP-2 derivative
  MISC_FEATURE (1): Xaa is imidazoacetyldeshistidine
XGDGSFSDEMNTILDNLAARDFINWLIQTRITDC

SEQ ID NO: 7 - protein, 34 aa, Artificial Sequence
  GLP-2 derivative
  MISC_FEATURE (1): Xaa is imidazoacetyldeshistidine
  MISC_FEATURE (2): Xaa is Aib(2-aminoisobutyric acid)
XXDGSFSDEMNTILDNLAARDFINWLIQTKITDC

SEQ ID NO: 8 - protein, 34 aa, Artificial Sequence
  GLP-2 derivative
  MISC_FEATURE (2): Xaa is Aib(2-aminoisobutyric acid)
HXDGSFSDEMNTILDNLAARDFINWLIQTKITDC

SEQ ID NO: 9 - protein, 34 aa, Artificial Sequence
  GLP-2 derivative
  MISC_FEATURE (1): Xaa = Histidine, imidazoacetyldeshistidine, desaminohistidine, beta-hydroxyimidazopropionyldeshistidine, N-dimethylhistidine, or beta-carboxyimidazopropionyldeshistidine
  MISC_FEATURE (2): Xaa is Alanine, Glycine, or Aib(2-aminoisobutyric acid)
  MISC_FEATURE (30): Xaa is Lysine, or Arginine
  MISC_FEATURE (34): Xaa is absent, Lysine, Arginine, Glutamine, Histidine, 6-azidolysine, or Cysteine
XXDGSFSDEMNTILDNLAARDFINWLIQTXITDX

SEQ ID NO: 10 - protein, 34 aa, Artificial Sequence; identical to SEQ ID NO: 9
  GLP-2 derivative
  MISC_FEATURE (1): Xaa = Histidine, imidazoacetyldeshistidine, desaminohistidine, beta-hydroxyimidazopropionyldeshistidine, N-dimethylhistidine, or beta-carboxyimidazopropionyldeshistidine
  MISC_FEATURE (2): Xaa is Alanine, Glycine, or Aib(2-aminoisobutyric acid)
  MISC_FEATURE (30): Xaa is Lysine, or Arginine
  MISC_FEATURE (34): Xaa = any one or more amino acid or any one or more amino acid which is modified

SEQ ID NO: 11 - protein, 12 aa, HOMO SAPIENS
ESKYGPPCPSCP

SEQ ID NO: 12 - protein, 11 aa, Artificial Sequence
  Variant of hinge region
ESKYGPPPSCP

SEQ ID NO: 13 - protein, 11 aa, Artificial Sequence
  Variant of hinge region
ESKYGPPCPSP

SEQ ID NO: 14 - protein, 10 aa, Artificial Sequence
  Variant of hinge region
ESKYGPPCPS

SEQ ID NO: 15 - protein, 10 aa, Artificial Sequence
  Variant of hinge region
ESKYGPPCPP

SEQ ID NO: 16 - protein, 8 aa, Artificial Sequence
  Variant of hinge region
KYGPPCPS

SEQ ID NO: 17 - protein, 8 aa, Artificial Sequence
  Variant of hinge region
ESKYGPPC

SEQ ID NO: 18 - protein, 7 aa, Artificial Sequence
  Variant of hinge region
EKYGPPC

SEQ ID NO: 19 - protein, 6 aa, Artificial Sequence
  Variant of hinge region
ESPSCP

SEQ ID NO: 20 - protein, 5 aa, Artificial Sequence
  Variant of hinge region
EPSCP

SEQ ID NO: 21 - protein, 4 aa, Artificial Sequence
  Variant of hinge region
PSCP

SEQ ID NO: 22 - protein, 10 aa, Artificial Sequence
  Variant of hinge region
ESKYGPPSCP

SEQ ID NO: 23 - protein, 9 aa, Artificial Sequence
  Variant of hinge region
KYGPPPSCP

SEQ ID NO: 24 - protein, 9 aa, Artificial Sequence
  Variant of hinge region
ESKYGPSCP

SEQ ID NO: 25 - protein, 8 aa, Artificial Sequence
  Variant of hinge region
ESKYGPPC

SEQ ID NO: 26 - protein, 7 aa, Artificial Sequence
  Variant of hinge region
KYGPPCP

SEQ ID NO: 27 - protein, 7 aa, Artificial Sequence
  Variant of hinge region
ESKPSCP

SEQ ID NO: 28 - protein, 6 aa, Artificial Sequence
  Variant of hinge region
ESPSCP

SEQ ID NO: 29 - protein, 4 aa, Artificial Sequence
  Variant of hinge region
EPSC

SEQ ID NO: 30 - protein, 3 aa, Artificial Sequence
  Variant of hinge region
SCP

SEQ ID NO: 31 - protein, 221 aa, homo sapiens
PSCPAPEFLGGPSVFLFPPKPKDTLMISRTPEVTCVVVDVSQEDPEVQFNWYVDGVEVHNAKTKPREEQFNSTYRVVSVLTVLHQDWLNGKEYKCKVSNKGLPSSIEKTISKAKGQPREPQVYTLPPSQEEMTKNQVSLTCLVKGFYPSDIAVEWESNGQPENNYKTTPPVLDSDGSFFLYSRLTVDKSRWQEGNVFSCSVMHEALHNHYTQKSLSLSLGK

SEQ ID NO: 32 - protein, 31 aa, Artificial Sequence
  GLP-1(7-37)
HAEGTFTSDVSSYLEGQAAKEFIAWLVKGRG

SEQ ID NO: 33 - protein, 39 aa, Artificial Sequence
  Exendin-3
HSDGTFTSDLSKQMEEEAVRLFIEWLKNGGPSSGAPPPS

SEQ ID NO: 34 - protein, 39 aa, Artificial Sequence
  Exendin-4
HGEGTFTSDLSKQMEEEAVRLFIEWLKNGGPSSGAPPPS

SEQ ID NO: 35 - protein, 442 aa, Homo sapiens
  MISC_FEATURE (1)..(442): Amino acids at position 1 to 442 form Human Immunoglobulin G4 Fc Fragment (homodimer)
  MISC_FEATURE (1)..(221): Amino acids at position 1 to 221 form one monomer
  MISC_FEATURE (222)..(442): Amino acids at position 222 to 442 form one monomer
  DISULFID (3)..(224): Amino acids at position 3 and position 224 form an inter-disulfide bond
  DISULFID (35)..(95): Amino acids at position 35 and position 95 form an intra-chain disulfide bond
  DISULFID (141)..(199): Amino acids at position 141 and position 199 form an intra-chain disulfide bond
  DISULFID (256)..(316): Amino acids at position 256 and position 316 form an intra-chain disulfide bond
  DISULFID (362)..(420): Amino acids at position 362 and position 420 form an intra-chain disulfide bond
PSCPAPEFLGGPSVFLFPPKPKDTLMISRTPEVTCVVVDVSQEDPEVQFNWYVDGVEVHNAKTKPREEQFNSTYRVVSVLTVLHQDWLNGKEYKCKVSNKGLPSSIEKTISKAKGQPREPQVYTLPPSQEEMTKNQVSLTCLVKGFYPSDIAVEWESNGQPENNYKTTPPVLDSDGSFFLYSRLTVDKSRWQEGNVFSCSVMHEALHNHYTQKSLSLSLGKPSCPAPEFLGGPSVFLFPPKPKDTLMISRTPEVTCVVVDVSQEDPEVQFNWYVDGVEVHNAKTKPREEQFNSTYRVVSVLTVLHQDWLNGKEYKCKVSNKGLPSSIEKTISKAKGQPREPQVYTLPPSQEEMTKNQVSLTCLVKGFYPSDIAVEWESNGQPENNYKTTPPVLDSDGSFFLYSRLTVDKSRWQEGNVFSCSVMHEALHNHYTQKSLSLSLGK